European Patent Application EP 4 245 858 A1, published September 20, 2023. Title: METHOD FOR DETECTING HUMAN MICROSATELLITE INSTABILITY site , AND USE THEREOF. Applicant: JIANG, Ying; HUANG, Xin. The sequence listing filed with the application follows.

SEQUENCE LISTING (50 sequences)

SEQ ID NO: 1 - DNA, 273 bp, Homo sapiens
ctcccctcgcttccaatgaatctcttcactctaggagaaagaatgacgagaacataacactagagacagtttgccatgaccccaagctcccctaccatgactttattctggaagatgctgcttctccaaagtgcattatgaaggaaaaaaaaaagcctggtgagactttcttcatgtgttcctgtagctctgatgagtgcaatgacaacatcatcttctcagaaggtgagttttcttctcttaagggtgtgggacctgagatctgtgccaatt

SEQ ID NO: 2 - DNA, 220 bp, Homo sapiens
ccagagtttagctcctcagaggtccctagcagcacgactgacatagcatctttctagtctgccgtaagtaccactacctttacacctcattgagaggcacttttttttttttttttttttgagatggagtcttgctctgtcaccccggctgcagtgcaatggcacatctcagctcactgcaacctccgcctcccaggttcaagtgattctcctgcctcag

SEQ ID NO: 3 - DNA, 221 bp, Homo sapiens
gcctgtagcagaattgcttgaacctgggaggcagaagttgcagtgacccaaaaccacaccactgcactccagcatgggcgacagagcaagactgtgtctcaaaaaaaaaaaaaaaaaaaaagtacctcaaaaatactctcctagggacctcaagtcttttccttctttaactgcttataaacatgcaaaaatggtccagtaagtctacaagtatttcacat

SEQ ID NO: 4 - DNA, 218 bp, Homo sapiens
aagggccctccttgggctgggggatgggccgggggtggggaggatgaggggtccctggaaatccagggtgaagatagaagtctggattatgttctaaatcttttttttttttttttttctccaaggagagaaaacagagcttcatgggaaacagcggcaacagttggtaagtagcagggccttccaggctgggatgggtgcagtgaggccaggcaggt

SEQ ID NO: 5 - DNA, 218 bp, Homo sapiens
agatgatggccaccctaagttcaggtggagagaatggggtttcttctttaaaaacccttctctcacaagaatttgcttctcaaattggagctgcagccaattttttttttttttttttggagacagggtctctgtcgcccaggctggagggcaatggagcgactgatcacggctcactgcagcctcaatctccctgggctcaggttatccttctacct

SEQ ID NO: 6 - DNA, 142 bp, Homo sapiens
atcagcagcatgaagtccagctaatacagtgcttgaacatgtaatatctcaaatctgtaatgtactttttttttttttaaggagcaaagaatctgcagagtgttgtgcttagtaaaatgaattttgaatcttttgtaaaaga

SEQ ID NO: 7 - DNA, 220 bp, Homo sapiens
cattttgagtattatatcaggcactatacagatcactttacacatattaactcatttaatttgttagtaccatggggttctgtcctgtttatcaagtccatttttttttttttttttttttaactttaaattctgggatacatgtgcagaacatgcaggtttgttacataggtatatctgtgccatggtggtatgctgcacctatcaacccgtcagctag

SEQ ID NO: 8 - DNA, 220 bp, Homo sapiens
gtgcctgtaatcctagcactttgggaggctgaggagggaggattgcttgagaccaagagttcaaggccaatcaagccaacatagtgagacccgtctctttaaaaaaaaaaaaaaaaaaaaggaagcatatgttcagtttctaaagttaatttacaggagaatgaaaaaactttaaaggttctgtggtgctcccctatcatagagggcaaggtacgatggt

SEQ ID NO: 9 - DNA, 221 bp, Homo sapiens
aggttatacatctaggaagaaacaagtcctacctaaacatatccttccttcccctcccaaaagttccccttcccagccttttatgcctctaacttagacctttttttttttttttttttttgagacagattttgctcagccgcccaggctggagtgcagcagcacgatctcagctcactacaaccaccacctcctgggttcaagggattctcccgtctcag

SEQ ID NO: 10 - DNA, 219 bp, Homo sapiens
ttttatttaaaataaagtctaaaatttcttagcatggcctgtatttctcatctctgacgtgccctcccccacttactcctgaccctctaccctagttgactttttttttttttttttttgagacagagtctgactctgttgcccaggctggaatgcagaagtgtgatcccggctcacagcaacccctgcctcccgggttcaagtgattctcctgtctca

SEQ ID NO: 11 - DNA, 20 bp, Artificial Sequence
  site 1 primer
agtttgccatgaccccaagc

SEQ ID NO: 12 - DNA, 23 bp, Artificial Sequence
  site 1 primer
actcatcagagctacaggaacac

SEQ ID NO: 13 - DNA, 23 bp, Artificial Sequence
  site 6 primer
tgaagtccagctaatacagtgct

SEQ ID NO: 14 - DNA, 24 bp, Artificial Sequence
  site 6 primer
attttactaagcacaacactctgc

SEQ ID NO: 15 - DNA, 20 bp, Artificial Sequence
  site 7 primer
ccatggggttctgtcctgtt

SEQ ID NO: 16 - DNA, 20 bp, Artificial Sequence
  site 7 primer
cagcataccaccatggcaca

SEQ ID NO: 17 - DNA, 20 bp, Artificial Sequence
  site 8 primer
gccaacatagtgagacccgt

SEQ ID NO: 18 - DNA, 20 bp, Artificial Sequence
  site 8 primer
tgataggggagcaccacaga

SEQ ID NO: 19 - DNA, 21 bp, Artificial Sequence
  site 2 primer
agcacgactgacatagcatct

SEQ ID NO: 20 - DNA, 20 bp, Artificial Sequence
  site 2 primer
gggtgacagagcaagactcc

SEQ ID NO: 21 - DNA, 20 bp, Artificial Sequence
  site 9 primer
tccttccttcccctcccaaa

SEQ ID NO: 22 - DNA, 20 bp, Artificial Sequence
  site 9 primer
gcggctgagcaaaatctgtc

SEQ ID NO: 23 - DNA, 20 bp, Artificial Sequence
  site 3 primer
gcagtgacccaaaaccacac

SEQ ID NO: 24 - DNA, 21 bp, Artificial Sequence
  site 3 primer
acttgaggtccctaggagagt

SEQ ID NO: 25 - DNA, 23 bp, Artificial Sequence
  site 4 primer
ccagggtgaagatagaagtctgg

SEQ ID NO: 26 - DNA, 20 bp, Artificial Sequence
  site 4 primer
acttaccaactgttgccgct

SEQ ID NO: 27 - DNA, 20 bp, Artificial Sequence
  site 10 primer
cctcccccacttactcctga

SEQ ID NO: 28 - DNA, 20 bp, Artificial Sequence
  site 10 primer
ccgggatcacacttctgcat

SEQ ID NO: 29 - DNA, 24 bp, Artificial Sequence
  site 5 primer
aacccttctctcacaagaatttgc

SEQ ID NO: 30 - DNA, 20 bp, Artificial Sequence
  site 5 primer
gtgatcagtcgctccattgc

SEQ ID NO: 31 - DNA, 24 bp, Artificial Sequence
  site 1 probe
caccaggcttttttttttccttca

SEQ ID NO: 32 - DNA, 22 bp, Artificial Sequence
  site 1 probe
cagcatcttccagaataaagtc

SEQ ID NO: 33 - DNA, 25 bp, Artificial Sequence
  site 6 probe
taatgtactttttttttttttaagg

SEQ ID NO: 34 - DNA, 19 bp, Artificial Sequence
  site 6 probe
catgtaatatctcaaatct

SEQ ID NO: 35 - DNA, 37 bp, Artificial Sequence
  site 7 probe
tcaagtccatttttttttttttttttttttaacttta

SEQ ID NO: 36 - DNA, 23 bp, Artificial Sequence
  site 7 probe
atacatgtgcagaacatgcaggt

SEQ ID NO: 37 - DNA, 37 bp, Artificial Sequence
  site 8 probe
atgcttccttttttttttttttttttttaaagagacg

SEQ ID NO: 38 - DNA, 19 bp, Artificial Sequence
  site 8 probe
cattctcctgtaaattaac

SEQ ID NO: 39 - DNA, 37 bp, Artificial Sequence
  site 2 probe
ttgagaggcacttttttttttttttttttttgagatg

SEQ ID NO: 40 - DNA, 17 bp, Artificial Sequence
  site 2 probe
agtcttgctctgtcacc

SEQ ID NO: 41 - DNA, 38 bp, Artificial Sequence
  site 9 probe
acttagacctttttttttttttttttttttgagacaga

SEQ ID NO: 42 - DNA, 17 bp, Artificial Sequence
  site 9 probe
ttgctcagccgcccagg

SEQ ID NO: 43 - DNA, 37 bp, Artificial Sequence
  site 3 probe
ttgaggtactttttttttttttttttttttgagacac

SEQ ID NO: 44 - DNA, 19 bp, Artificial Sequence
  site 3 probe
ttgctctgtcgcccatgct

SEQ ID NO: 45 - DNA, 38 bp, Artificial Sequence
  site 4 probe
tctaaatcttttttttttttttttttctccaaggagag

SEQ ID NO: 46 - DNA, 21 bp, Artificial Sequence
  site 4 probe
aaacagagcttcatgggaaac

SEQ ID NO: 47 - DNA, 38 bp, Artificial Sequence
  site 10 probe
ccctagttgactttttttttttttttttttgagacaga

SEQ ID NO: 48 - DNA, 20 bp, Artificial Sequence
  site 10 probe
tgactctgttgcccaggctg

SEQ ID NO: 49 - DNA, 38 bp, Artificial Sequence
  site 5 probe
caaattggagctgcagccaatttttttttttttttttt

SEQ ID NO: 50 - DNA, 18 bp, Artificial Sequence
  site 5 probe
cctgggcgacagagaccc